European Patent Application EP 4 365 298 A1, published May 8, 2024. Title: Method for producing negative-sense RNA virus vector and the produced netagive-sense RNA virus vector. Applicant: Regenerative Medicine iPS Gateway Center Co.,Ltd. The sequence listing filed with the application follows.

SEQUENCE LISTING (42 sequences)

SEQ ID NO: 1 - DNA, 1179 bp, Artificial Sequence
  EF1alpha
ggctccggtgcccgtcagtgggcagagcgcacatcgcccacagtccccgagaagttggggggaggggtcggcaattgaaccggtgcctagagaaggtggcgcggggtaaactgggaaagtgatgtcgtgtactggctccgcctttttcccgagggtgggggagaaccgtatataagtgcagtagtcgccgtgaacgttctttttcgcaacgggtttgccgccagaacacaggtaagtgccgtgtgtggttcccgcgggcctggcctctttacgggttatggcccttgcgtgccttgaattacttccacctggctgcagtacgtgattcttgatcccgagcttcgggttggaagtgggtgggagagttcgaggccttgcgcttaaggagccccttcgcctcgtgcttgagttgaggcctggcctgggcgctggggccgccgcgtgcgaatctggtggcaccttcgcgcctgtctcgctgctttcgataagtctctagccatttaaaatttttgatgacctgctgcgacgctttttttctggcaagatagtcttgtaaatgcgggccaagatctgcacactggtatttcggtttttggggccgcgggcggcgacggggcccgtgcgtcccagcgcacatgttcggcgaggcggggcctgcgagcgcggccaccgagaatcggacgggggtagtctcaagctggccggcctgctctggtgcctggcctcgcgccgccgtgtatcgccccgccctgggcggcaaggctggcccggtcggcaccagttgcgtgagcggaaagatggccgcttcccggccctgctgcagggagctcaaaatggaggacgcggcgctcgggagagcgggcgggtgagtcacccacacaaaggaaaagggcctttccgtcctcagccgtcgcttcatgtgactccacggagtaccgggcgccgtccaggcacctcgattagttctcgagcttttggagtacgtcgtctttaggttggggggaggggttttatgcgatggagtttccccacactgagtgggtggagactgaagttaggccagcttggcacttgatgtaattctccttggaatttgccctttttgagtttggatcttggttcattctcaagcctcagacagtggttcaaagtttttttcttccatttcaggtgtcgtga

SEQ ID NO: 2 - DNA, 1676 bp, Artificial Sequence
  CAG promoter
gacattgattattgactagttattaatagtaatcaattacggggtcattagttcatagcccatatatggagttccgcgttacataacttacggtaaatggcccgcctggctgaccgcccaacgacccccgcccattgacgtcaataatgacgtatgttcccatagtaacgccaatagggactttccattgacgtcaatgggtggagtatttacggtaaactgcccacttggcagtacatcaagtgtatcatatgccaagtacgccccctattgacgtcaatgacggtaaatggcccgcctggcattatgcccagtacatgaccttatgggactttcctacttggcagtacatctacgtattagtcatcgctattaccatggtcgaggtgagccccacgttctgcttcactctccccatctcccccccctccccacccccaattttgtatttatttattttttaattattttgtgcagcgatgggggcggggggggggggggggcgcgcgccaggcggggcggggcggggcgaggggcggggcggggcgaggcggagaggtgcggcggcagccaatcagagcggcgcgctccgaaagtttccttttatggcgaggcggcggcggcggcggccctataaaaagcgaagcgcgcggcgggcgggagtcgctgcgcgctgccttcgccccgtgccccgctccgccgccgcctcgcgccgcccgccccggctctgactgaccgcgttactcccacaggtgagcgggcgggacggcccttctcctccgggctgtaattagcgcttggtttaatgacggcttgtttcttttctgtggctgcgtgaaagccttgaggggctccgggagggccctttgtgcggggggagcggctcggggggtgcgtgcgtgtgtgtgtgcgtggggagcgccgcgtgcggctccgcgctgcccggcggctgtgagcgctgcgggcgcggcgcggggctttgtgcgctccgcagtgtgcgcgaggggagcgcggccgggggcggtgccccgcggtgcggggggggctgcgaggggaacaaaggctgcgtgcggggtgtgtgcgtgggggggtgagcagggggtgtgggcgcgtcggtcgggctgcaaccccccctgcacccccctccccgagttgctgagcacggcccggcttcgggtgcggggctccgtacggggcgtggcgcggggctcgccgtgccgggcggggggtggcggcaggtgggggtgccgggcggggcggggccgcctcgggccggggagggctcgggggaggggcgcggcggcccccggagcgccggcggctgtcgaggcgcggcgagccgcagccattgccttttatggtaatcgtgcgagagggcgcagggacttcctttgtcccaaatctgtgcggagccgaaatctgggaggcgccgccgcaccccctctagcgggcgcggggcgaagcggtgcggcgccggcaggaaggaaatgggcggggagggccttcgtgcgtcgccgcgccgccgtccccttctccctctccagcctcggggctgtccgcggggggacggctgccttcgggggggacggggcagggcggggttcggcttctggcgtgtgaccggcggctctagagcctctgctaaccatgttcatgccttcttctttttcctacag

SEQ ID NO: 3 - DNA, 732 bp, Artificial Sequence
  EmGFP
atggtgagcaagggcgaggagctgttcaccggggtggtgcccatcctggtcgagctggacggcgacgtaaacggccacaagttcagcgtgtccggcgagggcgagggcgatgccacctacggcaagctgaccctgaagttcatctgcaccaccggcaagctgcccgtgccctggcccaccctcgtgaccaccttgacctacggcgtgcagtgcttcgcccgctaccccgaccacatgaagcagcacgacttcttcaagtccgccatgcccgaaggctacgtccaggagcgcaccatcttcttcaaggacgacggcaactacaagacccgcgccgaggtgaagttcgagggcgacaccctggtgaaccgcatcgagctgaagggcatcgacttcaaggaggacggcaacatcctggggcacaagctggagtacaactacaacagccacaaggtctatatcaccgccgacaagcagaagaacggcatcaaggtgaacttcaagacccgccacaacatcgaggacggcagcgtgcagctcgccgaccactaccagcagaacacccccatcggcgacggccccgtgctgctgcccgacaaccactacctgagcacccagtccgccctgagcaaagaccccaacgagaagcgcgatcacatggtcctgctggagttcgtgaccgccgccgggatcactctcggcatggacgagctgtacaagtaatgataaccctga

SEQ ID NO: 4 - RNA, 708 nt, Artificial Sequence
  EBV EBER
ccauaaagccuaggguguaaaacaccgaccgcgccaccagauggcacacgugggggaaaugaggguuagcauaggcaacccccgccuacacaccaacuauagcaaaccccgccccgucacggugacguagucugucuugaggagauguagacuuguagacacugcaaaaccucaggaccuacgcugcccuagagguuuugcuagggaggagacguguguggcuguagccacccgucccggguacaagucccggguggugaggacggugucugugguugucuucccagacucugcuuucugccgucuucggucaaguaccagcuggugguccgcauguuuugauccaaacuuuuguuuuaggauuuaugcauccauuaucccgcaguuccaccuaaacggggcuuaacguugcaucccagaagaugcacgcuuaaccccgccuacaaccgugacguagcuguuuaccagcauguauagaguuacgguucgcuacaucaaacaggacagccguugcccuagugguuucggacacaccgccaacgcucagugcggugcuaccgacccgaggucaagucccgggggaggagaagagaggcuucccgccuagagcauuugcaagucaggauucucuaaucccucugggagaaggguauucggcuuguccgcuauuuuuuuguggcuaguuuugcacccacaacauguaaaggg

SEQ ID NO: 5 - RNA, 57 nt, Artificial Sequence
  HIV TAR
ggucucucugguuagaccagaucugagccugggagcucucuggcuaacuagggaacc

SEQ ID NO: 6 - protein, 149 aa, Artificial Sequence
  Polio virus 2Apro
GFGHQNKAVYTAGYKICNYHLATQDDLQNAVNVMWSRDLLVTESRAQGTDSIARCNCNAGVYYCESRRKYYPVSFVGPTFQYMEANNYYPARYQSHMLIGHGFASPGDCGGILRCHHGVIGIITAGGEGLVAFSDIRDLYAYEEEAMEQ

SEQ ID NO: 7 - protein, 190 aa, Artificial Sequence
  Vaccinia virus E3L
MSKIYIDERSNAEIVCEAIKTIGIEGATAAQLTRQLNMEKREVNKALYDLQRSAMVYSSDDIPPRWFMTTEADEADADAMSDVIIDDVSREKSMREDHKSFDDVIPAKKIIDWKGANPVTVINEYCQITRRDWSFRIESVGPSNSPTFYACVDIDGRVFDKADGKSKRDAKNNAAKLAVDKLLGYVIIRF

SEQ ID NO: 8 - protein, 365 aa, Artificial Sequence
  Reovirus sigma 3
MEVCLPNGHQVVDLINNAFEGRVSIYSAQEGWDKTISAQPDMMVCGGAVVCMHCLGVVGSLQRKLKHLPHHRCNQQIRHQDYVDVQFADRVTAHWKRGMLSFVAQMHEMMNDVSPDDLDRVRTEGGSLVELNWLQVDPNSMFRSIHSSWTDPLQVVDDLDTKLDQYWTALNLMIDSSDLIPNFMMRDPSHAFNGVKLGGDARQTQFSRTFDSRSSLEWGVMVYDYSELEHDPSKGRAYRKELVTPARDFGHFGLSHYSRATTPILGKMPAVFSGMLTGNCKMYPFIKGTAKLKTVRKLVEAVNHAWGVEKIRYALGPGGMTGWYNRTMQQAPIVLTPAALTMFPDTIKFGDLNYPVMIGDPMILG

SEQ ID NO: 9 - protein, 504 aa, Artificial Sequence
  Human p58_IPK
MVAPGSVTSRLGSVFPFLLVLVDLQYEGAECGVNADVEKHLELGKKLLAAGQLADALSQFHAAVDGDPDNYIAYYRRATVFLAMGKSKAALPDLTKVIQLKMDFTAARLQRGHLLLKQGKLDEAEDDFKKVLKSNPSENEEKEAQSQLIKSDEMQRLRSQALNAFGSGDYTAAIAFLDKILEVCVWDAELRELRAECFIKEGEPRKAISDLKAASKLKNDNTEAFYKISTLYYQLGDHELSLSEVRECLKLDQDHKRCFAHYKQVKKLNKLIESAEELIRDGRYTDATSKYESVMKTEPSIAEYTVRSKERICHCFSKDEKPVEAIRVCSEVLQMEPDNVNALKDRAEAYLIEEMYDEAIQDYETAQEHNENDQQIREGLEKAQRLLKQSQKRDYYKILGVKRNAKKQEIIKAYRKLALQWHPDNFQNEEEKKKAEKKFIDIAAAKEVLSDPEMRKKFDDGEDPLDAESQQGGGGNPFHRSWNSWQGFNPFSSGGPFRFKFHFN

SEQ ID NO: 10 - protein, 88 aa, Artificial Sequence
  Vaccinia virus K3L
MLAFCYSLPNAGDVIKGRVYEKDYALYIYLFDYPHSEAILAESVKMHMDRYVEYRDKLVGKTVKVKVIRVDYTKGYIDVNYKRMCRHQ

SEQ ID NO: 11 - protein, 86 aa, Artificial Sequence
  HIV Tat
MEPVDPRLEPWKHPGSQPKTACTNCYCKKCCFHCQVCFITKALGISYGRKKRRQRRRPPQGSQTHQVSLSKQPTSQPRGDPTGPKE

SEQ ID NO: 12 - protein, 248 aa, Artificial Sequence
  HSV ICP34.5
MARRRRHRGPRRPRPPGPTGAVPTAQSQVTSTPNSEPAVRSAPAAAPPPPPAGGPPPSCSLLLRQWLHVPESASDDDDDDDWPDSPPPEPAPEARPTAAAPRPRPPPPGVGPGGGADPSHPPSRPFRLPPRLALRLRVTAEHLARLRLRRAGGEGAPEPPATPATPATPATPATPARVRFSPHVRVRHLVVWASAARLARRGSWARERADRARFRRRVAEAEAVIGPCLGPEARARALARGAGPANSV

SEQ ID NO: 13 - RNA, 108 nt, Artificial Sequence
  nc866
cgggucggaguuagcucaagcgguuaccuccucaugccggacuuucuaucuguccaucucugugcugggguucgagacccgcgggugcuuacugacccuuuuaugcaa

SEQ ID NO: 14 - RNA, 272 nt, Artificial Sequence
  Long nc886
gucgggacgcucuggccggugaggcgugcgcagucguugacgcucuagaccgugcaaaaggagagccuguaagccgggucggaguuagcucaagcgguuaccuccucaugccggacuuucuaucuguccaucucugugcugggguucgagacccgcgggugcuuacugacccuuuuaugcaacuuccaggcgcggcggcugcugcgguagcuuuuuuggccacuggccgcgcgcggcguaagcgguuaggcuggaaagcgaaagcauuaagu

SEQ ID NO: 15 - protein, 447 aa, Artificial Sequence
  NS5A
SGSWLRDVWDWICTVLADFKTWLQSKLLPRLPGVPFFSCQRGYKGVWRGDGIMYTTCPCGAQITGHVKNGSMRIVGPRTCSNTWHGTFPINAYTTGPCTPSPAPNYSRALWRVAAEEYVEVTRVGDFHYVTGMTTDNVKCPCQVPAPEFFTELDGVRLHRYAPACKPLLRDEVTFQVGLNQYTVGSQLPCEPEPDVTVVTSMLTDPSHITAEAARRRLARGSPPSLASSSASQLSALSLKATCTTHHGAPDTDLIEANLLWRQEMGGNITRVESENKIVILDSFEPLRAEEDEREVSVAAEILRKTRKFPAAMPVWARPDYNPPLLESWKNPDYVPPVVHGCPLPPTKAPPIPPPRRKRTVVLTESTVSSALAELATKTFGSSGSSAVDSGTATGPPDQASAEGDAGSDAESYSSMPPLEGEPGDPDLSDGSWSTVSEEASEDVVCC

SEQ ID NO: 16 - protein, 148 aa, Artificial Sequence
  NS5A (1-148)
SGSWLRDVWDWICTVLADFKTWLQSKLLPRLPGVPFFSCQRGYKGVWRGDGIMYTTCPCGAQITGHVKNGSMRIVGPRTCSNTWHGTFPINAYTTGPCTPSPAPNYSRALWRVAAEEYVEVTRVGDFHYVTGMTTDNVKCPCQVPAPE

SEQ ID NO: 17 - RNA, 172 nt, Artificial Sequence
  VAI RNA
gggcacucuuccguggucugguggauaaauucgcaaggguaucauggcggacgaccgggguucgaaccccggauccggccguccgccgugauccaugcgguuaccgcccgcgugucgaacccaggugugcgacgucagacaacgggggagcgcuccuuuuggcuuccuucca

SEQ ID NO: 18 - RNA, 172 nt, Artificial Sequence
  VAI (c.74U>V)
gggcacucuuccguggucugguggauaaauucgcaaggguaucauggcggacgaccgggguucgaaccccggavccggccguccgccgugauccaugcgguuaccgcccgcgugucgaacccaggugugcgacgucagacaacgggggagcgcuccuuuuggcuuccuucca

SEQ ID NO: 19 - RNA, 330 nt, Artificial Sequence
  VAI long
gucgggacgcucuggccggugaggcgugcgcagucguugacgcucuagaccgugcaaaaggagagccuguaagcgggcacucuuccguggucugguggauaaauucgcaaggguaucauggcggacgaccgggguucgaaccccggauccggccguccgccgugauccaugcgguuaccgcccgcgugucgaacccaggugugcgacgucagacaacgggggagcgcuccuuuuggcuuccuuccaggcgcggcggcugcugcgcuagcuuuuuuggccacuggccgcgcgcggcguaagcgguuaggcuggaaagcgaaagcauuaagu

SEQ ID NO: 20 - RNA, 330 nt, Artificial Sequence
  VAI long (c.74>V)
gucgggacgcucuggccggugaggcgugcgcagucguugacgcucuagaccgugcaaaaggagagccuguaagcgggcacucuuccguggucugguggauaaauucgcaaggguaucauggcggacgaccgggguucgaaccccggavccggccguccgccgugauccaugcgguuaccgcccgcgugucgaacccaggugugcgacgucagacaacgggggagcgcuccuuuuggcuuccuuccaggcgcggcggcugcugcgcuagcuuuuuuggccacuggccgcgcgcggcguaagcgguuaggcuggaaagcgaaagcauuaagu

SEQ ID NO: 21 - RNA, 478 nt, Artificial Sequence
  VAI-VAII
gcgcagucguugacgcucuagaccgugcaaaaggagagccuguaagcgggcacucuuccguggucugguggauaaauucgcaaggguaucauggcggacgaccgggguucgaaccccggauccggccguccgccgugauccaugcgguuaccgcccgcgugucgaacccaggugugcgacgucagacaacgggggagcgcuccuuuuggcuuccuuccaggcgcggcggcugcugcgcuagcuuuuuuggccacuggccgcgcgcggcguaagcgguuaggcuggaaagcgaaagcauuaaguggcucgcucccuguagccggaggguuauuuuccaaggguugagucgcaggacccccgguucgagucucgggccggccggacugcggcgaacggggguuugccuccccgucaugcaagaccccgcuugcaaauuccuccggaaacagggacgagccccuuuuuugcuuuucccaga

SEQ ID NO: 22 - RNA, 172 nt, Artificial Sequence
  VAI (c.74U>M)
gggcacucuuccguggucugguggauaaauucgcaaggguaucauggcggacgaccgggguucgaaccccggamccggccguccgccgugauccaugcgguuaccgcccgcgugucgaacccaggugugcgacgucagacaacgggggagcgcuccuuuuggcuuccuucca

SEQ ID NO: 23 - RNA, 330 nt, Artificial Sequence
  VAI long (c.74U>M)
gucgggacgcucuggccggugaggcgugcgcagucguugacgcucuagaccgugcaaaaggagagccuguaagcgggcacucuuccguggucugguggauaaauucgcaaggguaucauggcggacgaccgggguucgaaccccggamccggccguccgccgugauccaugcgguuaccgcccgcgugucgaacccaggugugcgacgucagacaacgggggagcgcuccuuuuggcuuccuuccaggcgcggcggcugcugcgcuagcuuuuuuggccacuggccgcgcgcggcguaagcgguuaggcuggaaagcgaaagcauuaagu

SEQ ID NO: 24 - RNA, 330 nt, Artificial Sequence
  VAI long (c.191C>D)
gucgggacgcucuggccggugaggcgugcgcagucguugacgcucuagaccgugcaaaaggagagccuguaagcgggcacucuuccguggucugguggauaaauucgcaaggguaucauggcggacgaccgggguucgaaccccggauccggccguccgccgugauccaugcgguuaccgcccgcgugucgaacccaggugugcgacgucagacaacgggggagcgcuccuuuuggcuuccuuccaggcgcggcggcugcugcgduagcuuuuuuggccacuggccgcgcgcggcguaagcgguuaggcuggaaagcgaaagcauuaagu

SEQ ID NO: 25 - RNA, 330 nt, Artificial Sequence
  VAI long (c.74U>V, c.191C>D)
gucgggacgcucuggccggugaggcgugcgcagucguugacgcucuagaccgugcaaaaggagagccuguaagcgggcacucuuccguggucugguggauaaauucgcaaggguaucauggcggacgaccgggguucgaaccccggavccggccguccgccgugauccaugcgguuaccgcccgcgugucgaacccaggugugcgacgucagacaacgggggagcgcuccuuuuggcuuccuuccaggcgcggcggcugcugcgduagcuuuuuuggccacuggccgcgcgcggcguaagcgguuaggcuggaaagcgaaagcauuaagu

SEQ ID NO: 26 - RNA, 330 nt, Artificial Sequence
  VAI long (c.74U>M, c.191C>G)
gucgggacgcucuggccggugaggcgugcgcagucguugacgcucuagaccgugcaaaaggagagccuguaagcgggcacucuuccguggucugguggauaaauucgcaaggguaucauggcggacgaccgggguucgaaccccggamccggccguccgccgugauccaugcgguuaccgcccgcgugucgaacccaggugugcgacgucagacaacgggggagcgcuccuuuuggcuuccuuccaggcgcggcggcugcugcgguagcuuuuuuggccacuggccgcgcgcggcguaagcgguuaggcuggaaagcgaaagcauuaagu

SEQ ID NO: 27 - protein, 106 aa, Artificial Sequence
  SeV 106 aa of the C-terminal of C protein
MLETLINKIYTGPLGEELVQTLYLRIWAMEETPESLKILQMREDIRDQVLKMKTERWLRTLIRGEKTKLKDFQKRYEEVHPYLMKEKVEQVIMEEAWSLAAHIVQE

SEQ ID NO: 28 - protein, 230 aa, Artificial Sequence
  Influenza virus NS1
MDSNTVSSFQVDCFLWHIRKQVVDQELSDAPFLDRLRRDQRSLRGRGNTLGLDIKAATHVGKQIVEKILKEESDEALKMTMASTPASRYITDMTIEELSRNWFMLMPKQKVEGPLCIRMDQAIMEKNIMLKANFSVIFDRLETLVLLRAFTEEGAIVGEISPLPSFPGHTIEDVKNAIGVLIGGLEWNDNTVRVSKNLQRFAWRSSNENGGPPLTPKQKRKMARTARPKV

SEQ ID NO: 29 - protein, 149 aa, Artificial Sequence
  HSV Us11
MSQTQPPAPVGPGDPDVYLKGVPSAGMHPRGVHAPRGHPRMISGPPQRGDNDQAAGQCGDSGLLRVGADTTISKPSEAVRPPTIPRTPRVPREPRVPRPPREPREPRVPRAPRDPRVPRDPRDPRQPRSPREPRTPRTPREPRTARGSV

SEQ ID NO: 30 - protein, 213 aa, Artificial Sequence
  E3K3 fusion protein
MIIDDVSREKSMREDHKSFDDVIPAKKIIDWKDANPVTVINEYCQITKRDWSFRIESVGPSNSPTFYACVDIDGRVFDKADGKSKRDAKNNAAKLAVDKLLGYVIIRFEGRGSLLTCGDVEENPGPLAFCYSLPNAGDVIKGRVYENDYALYIYLFDYPHSEAILAESVKMHMDRYVEYRDKLVGKTVKVKVIRVDYTKGYIDVNYKRMCRHQ

SEQ ID NO: 31 - protein, 231 aa, Artificial Sequence
  E3Y3 fusion protein
MIIDDVSREKSMREDHKSFDDVIPAKKIIDWKDANPVTVINEYCQITKRDWSFRIESVGPSNSPTFYACVDIDGRVFDKADGKSKRDAKNNAAKLAVDKLLGYVIIRFEGRGSLLTCGDVEENPGPLETLINKIYTGPLGEELVQTLYLRIWAMEETPESLKILQMREDIRDQVLKMKTERWLRTLIRGEKTKLKDFQKRYEEVHPYLMKEKVEQVIMEEAWSLAAHIVQE

SEQ ID NO: 32 - DNA, 912 bp, Artificial Sequence
  EmGFP-VAI (c.74U>A)
atggtgagcaagggcgaggagctgttcaccggggtggtgcccatcctggtcgagctggacggcgacgtaaacggccacaagttcagcgtgtccggcgagggcgagggcgatgccacctacggcaagctgaccctgaagttcatctgcaccaccggcaagctgcccgtgccctggcccaccctcgtgaccaccttgacctacggcgtgcagtgcttcgcccgctaccccgaccacatgaagcagcacgacttcttcaagtccgccatgcccgaaggctacgtccaggagcgcaccatcttcttcaaggacgacggcaactacaagacccgcgccgaggtgaagttcgagggcgacaccctggtgaaccgcatcgagctgaagggcatcgacttcaaggaggacggcaacatcctggggcacaagctggagtacaactacaacagccacaaggtctatatcaccgccgacaagcagaagaacggcatcaaggtgaacttcaagacccgccacaacatcgaggacggcagcgtgcagctcgccgaccactaccagcagaacacccccatcggcgacggccccgtgctgctgcccgacaaccactacctgagcacccagtccgccctgagcaaagaccccaacgagaagcgcgatcacatggtcctgctggagttcgtgaccgccgccgggatcactctcggcatggacgagctgtacaagtaatgataaccctgactgtaagcgggcactcttccgtggtctggtggataaattcgcaagggtatcatggcggacgaccggggttcgaaccccggaaccggccgtccgccgtgatccatgcggttaccgcccgcgtgtcgaacccaggtgtgcgacgtcagacaacgggggagcgctccttttggcttccttcca

SEQ ID NO: 33 - DNA, 1062 bp, Artificial Sequence
  EmGFP-VAI L (c.74U>A)
atggtgagcaagggcgaggagctgttcaccggggtggtgcccatcctggtcgagctggacggcgacgtaaacggccacaagttcagcgtgtccggcgagggcgagggcgatgccacctacggcaagctgaccctgaagttcatctgcaccaccggcaagctgcccgtgccctggcccaccctcgtgaccaccttgacctacggcgtgcagtgcttcgcccgctaccccgaccacatgaagcagcacgacttcttcaagtccgccatgcccgaaggctacgtccaggagcgcaccatcttcttcaaggacgacggcaactacaagacccgcgccgaggtgaagttcgagggcgacaccctggtgaaccgcatcgagctgaagggcatcgacttcaaggaggacggcaacatcctggggcacaagctggagtacaactacaacagccacaaggtctatatcaccgccgacaagcagaagaacggcatcaaggtgaacttcaagacccgccacaacatcgaggacggcagcgtgcagctcgccgaccactaccagcagaacacccccatcggcgacggccccgtgctgctgcccgacaaccactacctgagcacccagtccgccctgagcaaagaccccaacgagaagcgcgatcacatggtcctgctggagttcgtgaccgccgccgggatcactctcggcatggacgagctgtacaagtaatgataaccctgagtcgggacgctctggccggtgaggcgtgcgcagtcgttgacgctctagaccgtgcaaaaggagagcctgtaagcgggcactcttccgtggtctggtggataaattcgcaagggtatcatggcggacgaccggggttcgaaccccggaaccggccgtccgccgtgatccatgcggttaccgcccgcgtgtcgaacccaggtgtgcgacgtcagacaacgggggagcgctccttttggcttccttccaggcgcggcggctgctgcggtagcttttttggccactggccgcgcgcggcgtaagcggttaggctggaaagcgaaagcattaagt

SEQ ID NO: 34 - RNA, 264 nt, Artificial Sequence
  VAI (264bp) 74c3p
cuguaagcgggcacucuuccguggucugguggauaaauucgcaaggguaucauggcggacgaccgggguucgaaccccggacccggccguccgccgugauccaugcgguuaccgcccgcgugucgaacccaggugugcgacgucagacaacgggggagcgcuccuuuuggcuuccuuccaggcgcggcggcugcugcgguagcuuuuuuggccacuggccgcgcgcggcguaagcgguuaggcuggaaagcgaaagcauuaagu

SEQ ID NO: 35 - RNA, 246 nt, Artificial Sequence
  VAI (246bp) 74c5p
gucgggacgcucuggccggugaggcgugcgcagucguugacgcucuagaccgugcaaaaggagagccuguaagcgggcacucuuccguggucugguggauaaauucgcaaggguaucauggcggacgaccgggguucgaaccccggacccggccguccgccgugauccaugcgguuaccgcccgcgugucgaacccaggugugcgacgucagacaacgggggagcgcuccuuuuggcuuccuucca

SEQ ID NO: 36 - RNA, 46 nt, Artificial Sequence
  Hh-Rbz
uuggucugaugaguccgugaggacgaaacggagucuagacuccguc

SEQ ID NO: 37 - RNA, 90 nt, Artificial Sequence
  HDV-Rbz
gggucggcauggcaucuccaccuccucgcgguccgaccugggcauccgaaggaggacgcacguccacucggauggcuaagggagagccac

SEQ ID NO: 38 - DNA, 48 bp, Artificial Sequence
  T7 terminator
ctagcataaccccttggggcctctaaacgggtcttgaggggttttttg

SEQ ID NO: 39 - DNA, 20 bp, Artificial Sequence
  Forward primer for L gene amplification
tgggtcattccctgaccaga

SEQ ID NO: 40 - DNA, 20 bp, Artificial Sequence
  Reverse primer for L gene amplification
cagcttcgatcgttctgcac

SEQ ID NO: 41 - DNA, 18 bp, Artificial Sequence
  Forward primer for VAI amplification
atcgagccttatgacagc

SEQ ID NO: 42 - DNA, 24 bp, Artificial Sequence
  Reverse primer for VAI amplification
gatacccttgcgaatttatccacc